European Patent Specification EP 3 759 108 B1, published August 30, 2023. Title: POLYPROLIN-MIMETIKA DES PROLIN-ABGELEITETEN MODULS-15. Applicant: Forschungsverbund Berlin e.V. Universität zu Köln. The sequence listing filed with the application follows.

SEQUENCE LISTING (3 sequences)

SEQ ID NO: 1 - protein, 5 aa, Artificial Sequence
  proline rich sequence
FPPPP

SEQ ID NO: 2 - protein, 13 aa, Artificial Sequence
  Peptide ligand
SFEFPPPPTEDEL

SEQ ID NO: 3 - protein, 5 aa, Artificial Sequence
  flanking epitope
TEDEL